European Patent Specification EP 3 564 257 B1, published June 18, 2025. Title: MUTANT FRAGMENTS OF OspA AND METHODS AND USES RELATING THERETO. Applicant: Valneva Austria GmbH. The sequence listing filed with the application follows.

SEQUENCE LISTING (65 sequences)

SEQ ID NO: 1 - protein, 150 aa, Artificial Sequence
  S3hybD1
FNEKGEVSEKILTRSNGTTLEYSQMTDAENATKAVETLKNGIKLPGNLVGGKTKLTVTCGTVTLSKNISKSGEITVALNDTETTPADKKTGEWKSDTSTLTISKNSQKTKQLVFTKENTITVQNYNRAGNALEGSPAEIKDLAELCAALK

SEQ ID NO: 2 - protein, 52 aa, Borrelia valaisiana
FNEKGEVSEKILTRSNGTTLEYSQMTDAENATKAVETLKNGIKLPGNLVGGK

SEQ ID NO: 3 - protein, 98 aa, Borrelia garinii
TKLTVTCGTVTLSKNISKSGEITVALNDTETTPADKKTGEWKSDTSTLTISKNSQKTKQLVFTKENTITVQNYNRAGNALEGSPAEIKDLAELCAALK

SEQ ID NO: 4 - protein, 274 aa, Borrelia valaisiana
MKKYLLGIGLILALIACKQNVSSLDEKNSASVDLPGEMKVLVSKEKDKDGKYSLVATVDKVELKGTSDKNNGSGTLEGVKDDKSKVKLTISDDLGETKLETFKEDGTLVSRKVNFKDKSFTEEKFNEKGEVSEKILTRSNGTTLEYSQMTDAENATKAVETLKNGIKLPGNLVGGKTTLKITEGTVTLSKHIAKSGEVTVEINDTSSTPNTKKTGKWDARNSTLTIIVDSKNKTKLVFTKQDTITVQSYNPAGNKLEGTAVEIKTLQELKNALK

SEQ ID NO: 5 - protein, 273 aa, Borrelia burgdorferi
MKKYLLGIGLILALIACKQNVSSLDEKNSVSVDLPGEMKVLVSKEKNKDGKYDLIATVDKLELKGTSDKNNGSGVLEGVKADKSKVKLTISDDLGQTTLEVFKEDGKTLVSKKVTSKDKSSTEEKFNEKGEVSEKIITRADGTRLEYTGIKSDGSGKAKEVLKGYVLEGTLTAEKTTLVVKEGTVTLSKNISKSGEVSVELNDTDSSAATKKTAAWNSGTSTLTITVNSKKTKDLVFTKENTITVQQYDSNGTKLEGSAVEITKLDEIKNALK

SEQ ID NO: 6 - protein, 273 aa, Borrelia afzelii
MKKYLLGIGLILALIACKQNVSSLDEKNSASVDLPGEMKVLVSKEKDKDGKYSLKATVDKIELKGTSDKDNGSGVLEGTKDDKSKAKLTIADDLSKTTFELFKEDGKTLVSRKVSSKDKTSTDEMFNEKGELSAKTMTRENGTKLEYTEMKSDGTGKAKEVLKNFTLEGKVANDKVTLEVKEGTVTLSKEIAKSGEVTVALNDTNTTQATKKTGAWDSKTSTLTISVNSKKTTQLVFTKQDTITVQKYDSAGTNLEGTAVEIKTLDELKNALK

SEQ ID NO: 7 - protein, 274 aa, Borrelia garinii
MKKYLLGIGLILALIACKQNVSSLDEKNSVSVDLPGGMKVLVSKEKDKDGKYSLMATVEKLELKGTSDKSNGSGVLEGEKADKSKAKLTISQDLNQTTFEIFKEDGKTLVSRKVNSKDKSSTEEKFNDKGKLSEKVVTRANGTRLEYTEIKNDGSGKAKEVLKGFALEGTLTDGGETKLTVTEGTVTLSKNISKSGEITVALNDTETTPADKKTGEWKSDTSTLTISKNSQKPKQLVFTKENTITVQNYNRAGNALEGSPAEIKDLAELKAALK

SEQ ID NO: 8 - protein, 274 aa, Borrelia garinii
MKKYLLGIGLILALIACKQNVSSLDEKNSVSVDLPGGMKVLVSKEKDKDGKYSLMATVEKLELKGTSDKSNGSGVLEGEKADKSKAKLTISQDLNQTTFEIFKEDGKTLVSRKVNSKDKSSTEEKFNDKGKLSEKVVTRANGTRLEYTEIKNDGSGKAKEVLKGFALEGTLTDGGETKLTVTEGTVTLSKNISKSGEITVALNDTETTPADKKTGEWKSDTSTLTISKNSQKTKQLVFTKENTITVQNYNRAGNALEGSPAEIKDLAELKAALK

SEQ ID NO: 9 - protein, 273 aa, Borrelia bavariensis
MKKYLLGIGLILALIACKQNVSSLDEKNSVSVDLPGEMKVLVSKEKDKDGKYSLMATVDKLELKGTSDKSNGSGTLEGEKSDKSKAKLTISEDLSKTTFEIFKEDGKTLVSKKVNSKDKSSIEEKFNAKGELSEKTILRANGTRLEYTEIKSDGTGKAKEVLKDFALEGTLAADKTTLKVTEGTVVLSKHIPNSGEITVELNDSNSTQATKKTGKWDSNTSTLTISVNSKKTKNIVFTKEDTITVQKYDSAGTNLEGNAVEIKTLDELKNALK

SEQ ID NO: 10 - protein, 273 aa, Borrelia garinii
MKKYLLGIGLILALIACKQNVSSLDEKNSVSVDLPGGMKVLVSKEKDKDGKYSLMATVEKLELKGTSDKNNGSGTLEGEKTDKSKVKLTIAEDLSKTTFEIFKEDGKTLVSKKVTLKDKSSTEEKFNEKGEISEKTIVRANGTRLEYTDIKSDKTGKAKEVLKDFTLEGTLAADGKTTLKVTEGTVTLSKNISKSGEITVALDDTDSSGNKKSGTWDSGTSTLTISKNRTKTKQLVFTKEDTITVQNYDSAGTNLEGKAVEITTLKELKNALK

SEQ ID NO: 11 - protein, 274 aa, Borrelia garinii
MKKYLLGIGLILALIACKQNVSSLDEKNSVSVDLPGGMTVLVSKEKDKDGKYSLEATVDKLELKGTSDKNNGSGTLEGEKTDKSKVKSTIADDLSQTKFEIFKEDGKTLVSKKVTLKDKSSTEEKFNGKGETSEKTIVRANGTRLEYTDIKSDGSGKAKEVLKDFTLEGTLAADGKTTLKVTEGTVVLSKNILKSGEITAALDDSDTTRATKKTGKWDSKTSTLTISVNSQKTKNLVFTKEDTITVQRYDSAGTNLEGKAVEITTLKELKNALK

SEQ ID NO: 12 - protein, 274 aa, Borrelia garinii
MKKYLLGIGLILALIACKQNVSSLDEKNSVSVDLPGEMKVLVSKEKDKDGKYSLEATVDKLELKGTSDKNNGSGVLEGVKAAKSKAKLTIADDLSQTKFEIFKEDGKTLVSKKVTLKDKSSTEEKFNDKGKLSEKVVTRANGTRLEYTEIQNDGSGKAKEVLKSLTLEGTLTADGETKLTVEAGTVTLSKNISESGEITVELKDTETTPADKKSGTWDSKTSTLTISKNSQKTKQLVFTKENTITVQKYNTAGTKLEGSPAEIKDLEALKAALK

SEQ ID NO: 13 - protein, 16 aa, Borrelia burgdorferi
MKKYLLGIGLILALIA

SEQ ID NO: 14 - protein, 15 aa, Borrelia burgdorferi
MRLLIGFALALALIG

SEQ ID NO: 15 - protein, 20 aa, Escherichia coli
MKATKLVLGAVILGSTLLAG

SEQ ID NO: 16 - protein, 21 aa, Artificial Sequence
  LN1 peptide linker
GTSDKNNGSGSKEKNKDGKYS

SEQ ID NO: 17 - protein, 11 aa, Borrelia burgdorferi
GYVLEGTLTAE

SEQ ID NO: 18 - protein, 11 aa, Borrelia afzelii
NFTLEGKVAND

SEQ ID NO: 19 - protein, 148 aa, Artificial Sequence
  B. burgdorferi OspA 126-273 with replaced hLFA-like sequence
FNEKGEVSEKIITRADGTRLEYTGIKSDGSGKAKEVLKNFTLEGKVANDKTTLVVKEGTVTLSKNISKSGEVSVELNDTDSSAATKKTAAWNSGTSTLTITVNSKKTKDLVFTKENTITVQQYDSNGTKLEGSAVEITKLDEIKNALK

SEQ ID NO: 20 - protein, 148 aa, Borrelia afzelii
FNEKGELSAKTMTRENGTKLEYTEMKSDGTGKAKEVLKNFTLEGKVANDKVTLEVKEGTVTLSKEIAKSGEVTVALNDTNTTQATKKTGAWDSKTSTLTISVNSKKTTQLVFTKQDTITVQKYDSAGTNLEGTAVEIKTLDELKNALK

SEQ ID NO: 21 - protein, 149 aa, Borrelia garinii
FNDKGKLSEKVVTRANGTRLEYTEIKNDGSGKAKEVLKGFALEGTLTDGGETKLTVTEGTVTLSKNISKSGEITVALNDTETTPADKKTGEWKSDTSTLTISKNSQKPKQLVFTKENTITVQNYNRAGNALEGSPAEIKDLAELKAALK

SEQ ID NO: 22 - protein, 148 aa, Borrelia bavariensis
FNAKGELSEKTILRANGTRLEYTEIKSDGTGKAKEVLKDFALEGTLAADKTTLKVTEGTVVLSKHIPNSGEITVELNDSNSTQATKKTGKWDSNTSTLTISVNSKKTKNIVFTKEDTITVQKYDSAGTNLEGNAVEIKTLDELKNALK

SEQ ID NO: 23 - protein, 148 aa, Borrelia garinii
FNEKGEISEKTIVRANGTRLEYTDIKSDKTGKAKEVLKDFTLEGTLAADGKTTLKVTEGTVTLSKNISKSGEITVALDDTDSSGNKKSGTWDSGTSTLTISKNRTKTKQLVFTKEDTITVQNYDSAGTNLEGKAVEITTLKELKNALK

SEQ ID NO: 24 - protein, 149 aa, Borrelia garinii
FNGKGETSEKTIVRANGTRLEYTDIKSDGSGKAKEVLKDFTLEGTLAADGKTTLKVTEGTVVLSKNILKSGEITAALDDSDTTRATKKTGKWDSKTSTLTISVNSQKTKNLVFTKEDTITVQRYDSAGTNLEGKAVEITTLKELKNALK

SEQ ID NO: 25 - protein, 149 aa, Borrelia garinii
FNDKGKLSEKVVTRANGTRLEYTEIQNDGSGKAKEVLKSLTLEGTLTADGETKLTVEAGTVTLSKNISESGEITVELKDTETTPADKKSGTWDSKTSTLTISKNSQKTKQLVFTKENTITVQKYNTAGTKLEGSPAEIKDLEALKAALK

SEQ ID NO: 26 - DNA, 1029 bp, Artificial Sequence
  Lip-S4D1-S3hybD1-nt
atgaaagctactaaactggtactgggcgcggtaatcctgggttctactctgctggcaggttgctcaagcttcaatgctaagggcgaactgagcgaaaaaacgatcctgcgtgcgaatggcacccgtctggaatacaccgaaatcaaatccgatggtacgggcaaagcaaaggaagtcctgaaagattttgctctggaaggtaccctggcggccgacaaaaccacgctgaaggtgacgtgcggcaccgtggttctgagcaaacatattccgaactctggtgaaatcaccgttgaactgaacgatagcaattctacgcaggcaaccaaaaagacgggcaaatgggacagtaatacctccacgctgaccatttcagtcaactcgaaaaagaccaaaaatattgtgttcacgaaggaagatacgatcaccgttcaaaaatatgactccgcgggcaccaacctggaaggcaatgccgtcgaaatcaaaaccctggatgaactgtgtaacgccctgaagggtactagtgacaaaaacaatggctctggtagcaaagagaaaaacaaagatggcaagtactcattcaacgaaaaaggcgaagtgagcgaaaaaattctgacccgtagcaatggcaccaccctggaatatagccagatgaccgatgcagaaaatgcaaccaaagcagttgaaaccctgaaaaacggtattaaactgcctggtaatctggttggtggtaaaaccaaactgaccgttacctgtggcaccgttaccctgagcaaaaacattagcaaaagcggtgaaattaccgtggcactgaatgataccgaaaccacaccggcagacaaaaaaaccggtgaatggaaaagcgataccagcaccctgaccattagtaaaaatagccagaaaacaaaacagctggtgtttaccaaagaaaacaccattaccgtgcagaattataaccgtgcaggtaatgcactggaaggtagtccggcagaaattaaagatctggcagaactgtgtgcagccctgaaataa

SEQ ID NO: 27 - protein, 322 aa, Artificial Sequence
  Lip-S4D1-S3hybD1-aa
  LIPID (1)..(1)
CSSFNAKGELSEKTILRANGTRLEYTEIKSDGTGKAKEVLKDFALEGTLAADKTTLKVTCGTVVLSKHIPNSGEITVELNDSNSTQATKKTGKWDSNTSTLTISVNSKKTKNIVFTKEDTITVQKYDSAGTNLEGNAVEIKTLDELCNALKGTSDKNNGSGSKEKNKDGKYSFNEKGEVSEKILTRSNGTTLEYSQMTDAENATKAVETLKNGIKLPGNLVGGKTKLTVTCGTVTLSKNISKSGEITVALNDTETTPADKKTGEWKSDTSTLTISKNSQKTKQLVFTKENTITVQNYNRAGNALEGSPAEIKDLAELCAALK

SEQ ID NO: 28 - DNA, 1020 bp, Artificial Sequence
  Lip-S1D1-S2D1-nt
atgaaagctactaaactggtactgggcgcggtaatcctgggttctactctgctggcaggttgctcaagcttcaacgaaaagggcgaagtcagcgaaaaaatcattacccgcgcagacggcacccgcctggaatacaccggcatcaaatcggacggcagcggcaaagcgaaagaagttctgaaaaactttaccctggaaggcaaagtcgcaaatgataaaaccaccctggtggtgaaatgcggcaccgttacgctgagcaaaaacattagtaaatccggtgaagtctctgtggaactgaatgataccgacagctctgcggccaccaagaaaaccgcagcttggaactcaggcacctcgacgctgaccattacggttaatagcaagaaaaccaaagatctggtcttcacgaaagaaaacaccatcacggtgcagcaatatgacagcaatggtaccaaactggaaggctccgctgtggaaatcacgaaactggatgaaatctgtaatgctctgaaaggtactagtgacaaaaacaatggctctggtagcaaagagaaaaacaaagatggcaagtactcattcaacgaaaaaggcgaactgtcggcgaaaacgatgacgcgtgaaaacggcaccaaactggaatatacggaaatgaaaagcgatggcaccggtaaagcgaaagaagttctgaaaaactttaccctggaaggcaaagtcgccaatgacaaagtcaccctggaagtgaaatgcggcaccgttacgctgtcaaaagaaattgcaaaatcgggtgaagtgaccgttgctctgaacgatacgaataccacgcaagcgaccaagaaaaccggcgcctgggacagcaaaacctctacgctgaccattagtgttaatagcaagaaaaccacgcagctggtcttcaccaaacaagatacgatcaccgtgcagaaatacgacagtgcgggtaccaacctggaaggcacggctgttgaaatcaaaaccctggacgaactgtgtaacgccctgaaa

SEQ ID NO: 29 - protein, 320 aa, Artificial Sequence
  Lip-S1D1-S2D1-aa
  LIPID (1)..(1)
CSSFNEKGEVSEKIITRADGTRLEYTGIKSDGSGKAKEVLKNFTLEGKVANDKTTLVVKCGTVTLSKNISKSGEVSVELNDTDSSAATKKTAAWNSGTSTLTITVNSKKTKDLVFTKENTITVQQYDSNGTKLEGSAVEITKLDEICNALKGTSDKNNGSGSKEKNKDGKYSFNEKGELSAKTMTRENGTKLEYTEMKSDGTGKAKEVLKNFTLEGKVANDKVTLEVKCGTVTLSKEIAKSGEVTVALNDTNTTQATKKTGAWDSKTSTLTISVNSKKTTQLVFTKQDTITVQKYDSAGTNLEGTAVEIKTLDELCNALK

SEQ ID NO: 30 - DNA, 1023 bp, Artificial Sequence
  Lip-S4D1-S3D1-nt
atgaaagctactaaactggtactgggcgcggtaatcctgggttctactctgctggcaggttgctcaagcttcaatgctaagggcgaactgagcgaaaaaacgatcctgcgtgcgaatggcacccgtctggaatacaccgaaatcaaatccgatggtacgggcaaagcaaaggaagtcctgaaagattttgctctggaaggtaccctggcggccgacaaaaccacgctgaaggtgacgtgcggcaccgtggttctgagcaaacatattccgaactctggtgaaatcaccgttgaactgaacgatagcaattctacgcaggcaaccaaaaagacgggcaaatgggacagtaatacctccacgctgaccatttcagtcaactcgaaaaagaccaaaaatattgtgttcacgaaggaagatacgatcaccgttcaaaaatatgactccgcgggcaccaacctggaaggcaatgccgtcgaaatcaaaaccctggatgaactgtgtaacgccctgaagggtactagtgacaaaaacaatggctctggtagcaaagagaaaaacaaagatggcaagtactcatttaacgataagggcaaactgtcggaaaaagtggtcacccgcgcaaatggcacccgcctggaatacacggaaatcaaaaacgatggtagcggcaaagcgaaggaagttctgaaaggctttgccctggaaggtaccctgacggatggcggtgaaaccaaactgaccgtgacgtgcggcaccgttacgctgtctaaaaacattagcaagtctggtgaaatcacggtcgcactgaatgataccgaaaccacgccggctgacaaaaagaccggcgaatggaaaagtgacacctccacgctgaccatttcaaagaactcgcagaaaccgaagcaactggtcttcaccaaagaaaacacgatcaccgtgcagaactataatcgtgccggtaatgctctggaaggctcaccggctgaaatcaaggacctggctgaactgtgtgcggcactgaaa

SEQ ID NO: 31 - protein, 321 aa, Artificial Sequence
  Lip-S4D1-S3D1-aa
  LIPID (1)..(1)
CSSFNAKGELSEKTILRANGTRLEYTEIKSDGTGKAKEVLKDFALEGTLAADKTTLKVTCGTVVLSKHIPNSGEITVELNDSNSTQATKKTGKWDSNTSTLTISVNSKKTKNIVFTKEDTITVQKYDSAGTNLEGNAVEIKTLDELCNALKGTSDKNNGSGSKEKNKDGKYSFNDKGKLSEKVVTRANGTRLEYTEIKNDGSGKAKEVLKGFALEGTLTDGGETKLTVTCGTVTLSKNISKSGEITVALNDTETTPADKKTGEWKSDTSTLTISKNSQKPKQLVFTKENTITVQNYNRAGNALEGSPAEIKDLAELCAALK

SEQ ID NO: 32 - DNA, 1023 bp, Artificial Sequence
  Lip-S5D1-S6D1-nt
atgaaagctactaaactggtactgggcgcggtaatcctgggttctactctgctggcaggttgctcaagcttcaacgaaaagggcgaaatctcagaaaaaaccatcgtccgcgctaacggcacccgcctggaatacaccgacatcaaatcagacaagaccggtaaagcgaaggaagttctgaaagattttacgctggaaggtaccctggcagcagacggtaaaaccacgctgaaggtgacctgcggtaccgttacgctgtccaaaaacattagtaagtccggcgaaatcacggtcgccctggatgacaccgatagctctggcaacaaaaagagcggtacctgggattcaggcacctcgacgctgaccatttctaaaaatcgtacgaaaaccaagcagctggtcttcacgaaagaagatacgatcaccgtgcaaaactatgacagcgcaggtaccaatctggaaggcaaagctgtggaaattaccacgctgaaagaactgtgtaatgctctgaaaggtactagtgacaaaaacaatggctctggtagcaaagagaaaaacaaagatggcaagtactcattcaacggcaaaggtgaaacgagcgaaaagaccatcgtgcgtgcgaacggtacccgcctggaatatacggacattaaatcggacggcagcggcaaagcaaaggaagtcctgaaagattttacgctggaaggtaccctggcagcagacggtaaaaccacgctgaaggtgacgtgcggcaccgtggttctgtcaaaaaacattctgaagtcgggtgaaatcaccgcagctctggatgacagcgataccacgcgtgctacgaaaaagaccggtaaatgggatagcaagacctctacgctgaccattagtgtcaactcccagaaaacgaagaatctggtgttcaccaaagaagatacgatcaccgttcaacgctatgacagtgcgggcaccaacctggaaggcaaagccgttgaaattaccacgctgaaagaactgtgtaatgctctgaaa

SEQ ID NO: 33 - protein, 321 aa, Artificial Sequence
  Lip-S5D1-S6D1-aa
  LIPID (1)..(1)
CSSFNEKGEISEKTIVRANGTRLEYTDIKSDKTGKAKEVLKDFTLEGTLAADGKTTLKVTCGTVTLSKNISKSGEITVALDDTDSSGNKKSGTWDSGTSTLTISKNRTKTKQLVFTKEDTITVQNYDSAGTNLEGKAVEITTLKELCNALKGTSDKNNGSGSKEKNKDGKYSFNGKGETSEKTIVRANGTRLEYTDIKSDGSGKAKEVLKDFTLEGTLAADGKTTLKVTCGTVVLSKNILKSGEITAALDDSDTTRATKKTGKWDSKTSTLTISVNSQKTKNLVFTKEDTITVQRYDSAGTNLEGKAVEITTLKELCNALK

SEQ ID NO: 34 - protein, 268 aa, Artificial Sequence
  B. burgdorferi  (strain B31, OspA serotype 1) aa 18-273
CSSFKQNVSSLDEKNSVSVDLPGEMKVLVSKEKNKDGKYDLIATVDKLELKGTSDKNNGSGVLEGVKADKSKVKLTISDDLGQTTLEVFKEDGKTLVSKKVTSKDKSSTEEKFNEKGEVSEKIITRADGTRLEYTGIKSDGSGKAKEVLKGYVLEGTLTAEKTTLVVKEGTVTLSKNISKSGEVSVELNDTDSSAATKKTAAWNSGTSTLTITVNSKKTKDLVFTKENTITVQQYDSNGTKLEGSAVEITKLDEIKNALKLEHHHHHH

SEQ ID NO: 35 - protein, 268 aa, Artificial Sequence
  B. afzelii (strain K78; OspA serotype 2) aa 18-273
CSSFKQNVSSLDEKNSASVDLPGEMKVLVSKEKDKDGKYSLKATVDKIELKGTSDKDNGSGVLEGTKDDKSKAKLTIADDLSKTTFELFKEDGKTLVSRKVSSKDKTSTDEMFNEKGELSAKTMTRENGTKLEYTEMKSDGTGKAKEVLKNFTLEGKVANDKVTLEVKEGTVTLSKEIAKSGEVTVALNDTNTTQATKKTGAWDSKTSTLTISVNSKKTTQLVFTKQDTITVQKYDSAGTNLEGTAVEIKTLDELKNALKLEHHHHHH

SEQ ID NO: 36 - protein, 269 aa, Artificial Sequence
  B. garinii (strain PBr; OspA serotype 3) aa 18-274
CSSFKQNVSSLDEKNSVSVDLPGGMKVLVSKEKDKDGKYSLMATVEKLELKGTSDKSNGSGVLEGEKADKSKAKLTISQDLNQTTFEIFKEDGKTLVSRKVNSKDKSSTEEKFNDKGKLSEKVVTRANGTRLEYTEIKNDGSGKAKEVLKGFALEGTLTDGGETKLTVTEGTVTLSKNISKSGEITVALNDTETTPADKKTGEWKSDTSTLTISKNSQKTKQLVFTKENTITVQNYNRAGNALEGSPAEIKDLAELKAALKLEHHHHHH

SEQ ID NO: 37 - protein, 268 aa, Artificial Sequence
  B. bavariensis (strain PBi; OspA serotype 4) aa 18-273
CSSFKQNVSSLDEKNSVSVDLPGEMKVLVSKEKDKDGKYSLMATVDKLELKGTSDKSNGSGTLEGEKSDKSKAKLTISEDLSKTTFEIFKEDGKTLVSKKVNSKDKSSIEEKFNAKGELSEKTILRANGTRLEYTEIKSDGTGKAKEVLKDFALEGTLAADKTTLKVTEGTVVLSKHIPNSGEITVELNDSNSTQATKKTGKWDSNTSTLTISVNSKKTKNIVFTKEDTITVQKYDSAGTNLEGNAVEIKTLDELKNALKLEHHHHHH

SEQ ID NO: 38 - protein, 268 aa, Artificial Sequence
  B. garinii (strain PHei; OspA serotype 5) aa 18-273
CSSFKQNVSSLDEKNSVSVDLPGGMKVLVSKEKDKDGKYSLMATVEKLELKGTSDKNNGSGTLEGEKTDKSKVKLTIAEDLSKTTFEIFKEDGKTLVSKKVTLKDKSSTEEKFNEKGEISEKTIVRANGTRLEYTDIKSDKTGKAKEVLKDFTLEGTLAADGKTTLKVTEGTVTLSKNISKSGEITVALDDTDSSGNKKSGTWDSGTSTLTISKNRTKTKQLVFTKEDTITVQNYDSAGTNLEGKAVEITTLKELKNALKLEHHHHHH

SEQ ID NO: 39 - protein, 269 aa, Artificial Sequence
  B. garinii (strain DK29; OspA serotype 6) aa 18-274
CSSFKQNVSSLDEKNSVSVDLPGGMTVLVSKEKDKDGKYSLEATVDKLELKGTSDKNNGSGTLEGEKTDKSKVKSTIADDLSQTKFEIFKEDGKTLVSKKVTLKDKSSTEEKFNGKGETSEKTIVRANGTRLEYTDIKSDGSGKAKEVLKDFTLEGTLAADGKTTLKVTEGTVVLSKNILKSGEITAALDDSDTTRATKKTGKWDSKTSTLTISVNSQKTKNLVFTKEDTITVQRYDSAGTNLEGKAVEITTLKELKNALKLEHHHHHH

SEQ ID NO: 40 - protein, 278 aa, Artificial Sequence
  Chimeric OspA Serotype1/Serotype2, N-terminal lipidation
MRLLIGFALALALIGCAQKGAESIGSVSVDLPGEMKVLVSKEKDKNGKYDLIATVDKLELKGTSDKNNGSGVLEGVKTNKSKVKLTISDDLGQTTLEVFKEDGKTLVSKKVTSKDKSSTEEKFNEKGEVSEKIITMADGTRLEYTGIKSDGTGKAKYVLKNFTLEGKVANDKTTLEVKEGTVTLSMNISKSGEVSVELNDTDSSAATKKTAAWNSKTSTLTISVNSKKTTQLVFTKQDTITVQKYDSAGTNLEGTAVEIKTLDELKNALKLEHHHHHH

SEQ ID NO: 41 - protein, 278 aa, Artificial Sequence
  Chimeric OspA Serotype5/Serotype3, N-terminal lipidation
MRLLIGFALALALIGCAQKGAESIGSVSVDLPGGMKVLVSKEKDKNGKYSLMATVEKLELKGTSDKNNGSGTLEGEKTNKSKVKLTIAEDLSKTTFEIFKEDGKTLVSKKVTLKDKSSTEEKFNEKGEISEKTIVMANGTRLEYTDIKSDKTGKAKYVLKDFTLEGTLAADGKTTLKVTEGTVTLSMNISKSGEITVALDDTDSSGNKKSGTWDSDTSTLTISKNSQKTKQLVFTKENTITVQNYNRAGNALEGSPAEIKDLAELKAALKLEHHHHHH

SEQ ID NO: 42 - protein, 279 aa, Artificial Sequence
  Chimeric OspA Serotype6/Serotype4, N-terminal lipidation
MRLLIGFALALALIGCAQKGAESIGSVSVDLPGGMTVLVSKEKDKNGKYSLEATVDKLELKGTSDKNNGSGTLEGEKTNKSKVKLTIADDLSQTKFEIFKEDAKTLVSKKVTLKDKSSTEEKFNEKGETSEKTIVMANGTRLEYTDIKSDGSGKAKYVLKDFTLEGTLAADGKTTLKVTEGTVVLSMNILKSGEITVALDDSDTTQATKKTGKWDSNTSTLTISVNSKKTKNIVFTKEDTITVQKYDSAGTNLEGNAVEIKTLDELKNALKLEHHHHHH

SEQ ID NO: 43 - protein, 148 aa, Artificial Sequence
  S1D1
FNEKGEVSEKIITRADGTRLEYTGIKSDGSGKAKEVLKNFTLEGKVANDKTTLVVKCGTVTLSKNISKSGEVSVELNDTDSSAATKKTAAWNSGTSTLTITVNSKKTKDLVFTKENTITVQQYDSNGTKLEGSAVEITKLDEICNALK

SEQ ID NO: 44 - protein, 148 aa, Artificial Sequence
  S2D1
FNEKGELSAKTMTRENGTKLEYTEMKSDGTGKAKEVLKNFTLEGKVANDKVTLEVKCGTVTLSKEIAKSGEVTVALNDTNTTQATKKTGAWDSKTSTLTISVNSKKTTQLVFTKQDTITVQKYDSAGTNLEGTAVEIKTLDELCNALK

SEQ ID NO: 45 - protein, 149 aa, Artificial Sequence
  S3D1
FNDKGKLSEKVVTRANGTRLEYTEIKNDGSGKAKEVLKGFALEGTLTDGGETKLTVTCGTVTLSKNISKSGEITVALNDTETTPADKKTGEWKSDTSTLTISKNSQKTKQLVFTKENTITVQNYNRAGNALEGSPAEIKDLAELCAALK

SEQ ID NO: 46 - protein, 148 aa, Artificial Sequence
  S4D1
FNAKGELSEKTILRANGTRLEYTEIKSDGTGKAKEVLKDFALEGTLAADKTTLKVTCGTVVLSKHIPNSGEITVELNDSNSTQATKKTGKWDSNTSTLTISVNSKKTKNIVFTKEDTITVQKYDSAGTNLEGNAVEIKTLDELCNALK

SEQ ID NO: 47 - protein, 148 aa, Artificial Sequence
  S5D1
FNEKGEISEKTIVRANGTRLEYTDIKSDKTGKAKEVLKDFTLEGTLAADGKTTLKVTCGTVTLSKNISKSGEITVALDDTDSSGNKKSGTWDSGTSTLTISKNRTKTKQLVFTKEDTITVQNYDSAGTNLEGKAVEITTLKELCNALK

SEQ ID NO: 48 - protein, 149 aa, Artificial Sequence
  S6D1
FNGKGETSEKTIVRANGTRLEYTDIKSDGSGKAKEVLKDFTLEGTLAADGKTTLKVTCGTVVLSKNILKSGEITAALDDSDTTRATKKTGKWDSKTSTLTISVNSQKTKNLVFTKEDTITVQRYDSAGTNLEGKAVEITTLKELCNALK

SEQ ID NO: 49 - protein, 150 aa, Artificial Sequence; identical to SEQ ID NO: 1
  S3HYBD1 (BVA)

SEQ ID NO: 50 - protein, 150 aa, Artificial Sequence
  BVAD1
FNEKGEVSEKILTRSNGTTLEYSQMTDAENATKAVETLKNGIKLPGNLVGGKTTLKITCGTVTLSKHIAKSGEVTVEINDTSSTPNTKKTGKWDARNSTLTIIVDSKNKTKLVFTKQDTITVQSYNPAGNKLEGTAVEIKTLQELCNALK

SEQ ID NO: 51 - protein, 148 aa, Artificial Sequence
  S3HYBD1 (BSP)
FNEKGELSEKTLVRANGTKLEYTEIKSDGTGKAKEVLKDFTLEGTLANEKTKLTVTCGTVTLSKNISKSGEITVALNDTETTPADKKTGEWKSDTSTLTISKNSQKTKQLVFTKENTITVQNYNRAGNALEGSPAEIKDLAELCAALK

SEQ ID NO: 52 - protein, 148 aa, Artificial Sequence
  MSPD1
FNEKGELSEKTLVRANGTKLEYTEIKSDGTGKAKEVLKDFTLEGTLANEKATLTVKCGTVTLSKNIDKSGEVTVALNDTDSTAATKKTGAWDSKTSTLTITVNSKKTKDLVFTKQDTITVQKYDSAGTTLEGSAVEIKTLDELCNALK

SEQ ID NO: 53 - DNA, 21 bp, Artificial Sequence
  Forward primer for the 16S-23S intergenic spacer
gtatgtttagtgaggggggtg

SEQ ID NO: 54 - DNA, 22 bp, Artificial Sequence
  Reverse primer for the 16S-23S intergenic spacer
ggatcatagctcaggtggttag

SEQ ID NO: 55 - DNA, 22 bp, Artificial Sequence
  Forward nested primer for the 16S-23S intergenic spacer
aggggggtgaagtcgtaacaag

SEQ ID NO: 56 - DNA, 22 bp, Artificial Sequence
  Reverse nested primer for the 16S-23S intergenic spacer
gtctgataaacctgaggtcgga

SEQ ID NO: 57 - DNA, 20 bp, Artificial Sequence
  Forward primer for the RecA gene of Borrelia
catgctcttgatcctgttta

SEQ ID NO: 58 - DNA, 20 bp, Artificial Sequence
  Reverse primer for the RecA gene of Borrelia
cccatttctccatctatctc

SEQ ID NO: 59 - protein, 25 aa, Artificial Sequence
  25-mer peptide from the Invariable Region 6 (IR6) of VlsE
MKKDDQIAAAMVLRGMAKDGQFALK

SEQ ID NO: 60 - protein, 36 aa, Artificial Sequence
  Mouse cathelin
RLAGLLRKGGEKIGEKLKKIGQKIKNFFQKLVPQPE

SEQ ID NO: 61 - protein, 11 aa, Artificial Sequence
  KLK peptide
KLKLLLLLKLK

SEQ ID NO: 62 - protein, 4 aa, Artificial Sequence
  N-terminal peptide for lipidation
CKQN

SEQ ID NO: 63 - DNA, 26 bp, Artificial Sequence
  5'-(dIdC)13-3'
  misc_feature (1)..(26): n=inosine
ncncncncncncncncncncncncnc

SEQ ID NO: 64 - protein, 8 aa, Artificial Sequence
  C-terminal His tag
LEHHHHHH

SEQ ID NO: 65 - protein, 4 aa, Artificial Sequence
  N-terminal CSSF for addition of lipids
CSSF